European Patent Specification EP 3 177 650 B1, published November 5, 2025. Title: ANTI-CERAMIDE ANTIBODIES. Applicant: MEMORIAL SLOAN KETTERING CANCER CENTER ROTOLO, Jimmy KOLESNICK, Richard. The sequence listing filed with the application follows.

SEQUENCE LISTING (45 sequences)

SEQ ID NO: 1 - protein, 10 aa, Artificial Sequence
  Synthetic: heavy chain variable region CDR1 of the anti-ceramide antibody
GYTFTDHTIH

SEQ ID NO: 2 - protein, 17 aa, Artificial Sequence
  Synthetic: heavy chain variable region CDR2
YNYPRDGSTKYNEKFKG

SEQ ID NO: 3 - protein, 11 aa, Artificial Sequence
  Synthetic: heavy chain variable region CDR3
GFITTVVPSAY

SEQ ID NO: 4 - protein, 11 aa, Artificial Sequence
  Synthetic: light chain variable region CDR1
RASKSISKYLA

SEQ ID NO: 5 - protein, 7 aa, Artificial Sequence
  Synthetic: light chain variable region CDR2
SGSTLQS

SEQ ID NO: 6 - protein, 9 aa, Artificial Sequence
  Synthetic: light chain variable region CDR3
QQHNEYPWT

SEQ ID NO: 7 - protein, 119 aa, Artificial Sequence
  Synthetic: heavy chain variable region sequence
QVQLQQSDAELVKPGASVKISCKVSGYTFTDHTIHWMKQRPEQGLEWIGYNPRDGSTKYNEKFGKATLTDADKSSSTAYMQLNSLTSEDSAVYFCAKGFITTVVPSAYWGQGTLVTVSA

SEQ ID NO: 8 - protein, 107 aa, Artificial Sequence
  Synthetic: light chain variable region sequence
DVQITQSPSYLAASPGETITINCRASKSISKYLAWYQEKPGKTNKLLIYSGSTLQSGIPSRFSGSGSGTDFTLTISSLEPEDFAMYYCQQHNEYPWTFGGGTKLEIK

SEQ ID NO: 9 - protein, 10 aa, Artificial Sequence
  Synthetic: heavy chain variable region CDR1
GYAFSSYWMN

SEQ ID NO: 10 - protein, 17 aa, Artificial Sequence
  Synthetic: heavy chain variable region CDR2
QIYPGDGDTNYNGKFKG

SEQ ID NO: 11 - protein, 10 aa, Artificial Sequence
  Synthetic: heavy chain variable region CDR3
RCYYGLYFDV

SEQ ID NO: 12 - protein, 11 aa, Artificial Sequence
  Synthetic: light chain variable region CDR1
KASQDINRYLS

SEQ ID NO: 13 - protein, 7 aa, Artificial Sequence
  Synthetic: light chain variable region CDR2
RANRLVD

SEQ ID NO: 14 - protein, 9 aa, Artificial Sequence
  Synthetic: light chain variable region CDR3
LQYDEFPYT

SEQ ID NO: 15 - protein, 119 aa, Artificial Sequence
  Synthetic: heavy chain variable region sequence
QVQLQQSGAELVKPGASVKISCKASGYAFSSYWMNWVKQRPGKGLEWIGQIYPGDGDTNYNGKFKGKATLTADKSSSTAYMQLSSLTSEDSAVYFCTRRCYYGLYFDVWGTGTTVTVSS

SEQ ID NO: 16 - protein, 108 aa, Artificial Sequence
  Synthetic: light chain variable region sequence
DIKMTQSPSSRYASLGERVTITCKASQDINRYLSWFQQKPGKSPKTLIYRANRLVDGVPSSRFSGSGSGQDYSLTISSLEYEDMGIYYCLQYDEFPYTFGGGTKLEIK

SEQ ID NO: 17 - protein, 10 aa, Artificial Sequence
  Synthetic: heavy chain variable region CDR1 of the anti-ceramide antibody
GYTFTSYWMH

SEQ ID NO: 18 - protein, 16 aa, Artificial Sequence
  Synthetic: heavy chain variable region CDR2
YINPSSGYTKYNQFKD

SEQ ID NO: 19 - protein, 8 aa, Artificial Sequence
  Synthetic: heavy chain variable region CDR3
GGYYGFAY

SEQ ID NO: 20 - protein, 10 aa, Artificial Sequence
  Synthetic: light chain variable region CDR1
SASSSVSYMY

SEQ ID NO: 21 - protein, 7 aa, Artificial Sequence
  Synthetic: light chain variable region CDR2
LTSNLAS

SEQ ID NO: 22 - protein, 9 aa, Artificial Sequence
  Synthetic: light chain variable region CDR3
QQWSSNPLT

SEQ ID NO: 23 - protein, 117 aa, Artificial Sequence
  Synthetic: heavy chain variable region sequence
QVQLQQSGAELAKPGASVKLSCKASGYTFTSYWMHWVKQRPGQGLEWIGYINPSSGYTKYNQKFKDKATLTADKSSSTAYMQLSSLTYEDSAVYYCARGGYYGFAYWGQGTLVTVSA

SEQ ID NO: 24 - protein, 106 aa, Artificial Sequence
  Synthetic: light chain variable region sequence
QIVLTQSPALMSASPGEKVTMTCSASSSVSYMYWYQQKPRSSPKPWIYLTSNLASGVPARFSGSGSGTSYSLTISSMEAEDAATYYCQQWSSNPLTFGAGTKLELK

SEQ ID NO: 25 - protein, 10 aa, Artificial Sequence
  Synthetic: heavy chain variable region CDR1 of the anti-ceramide antibody
GFSLTGYGVH

SEQ ID NO: 26 - protein, 16 aa, Artificial Sequence
  Synthetic: heavy chain variable region CDR2
VIWSGGSTDYNAAFIS

SEQ ID NO: 27 - protein, 10 aa, Artificial Sequence
  Synthetic: heavy chain variable region CDR3
NYGYDYAMDY

SEQ ID NO: 28 - protein, 11 aa, Artificial Sequence
  Synthetic: light chain variable region CDR1
RASQSIGTSIH

SEQ ID NO: 29 - protein, 7 aa, Artificial Sequence
  Synthetic: light chain variable region CDR2
YASESIS

SEQ ID NO: 30 - protein, 9 aa, Artificial Sequence
  Synthetic: light chain variable region CDR3
QQSNSWPFT

SEQ ID NO: 31 - protein, 116 aa, Artificial Sequence
  Synthetic: heavy chain variable region sequence
QVQLKQSGPGVQPSSLSITCTVSGFSLTSYGVHWVRQSPGKGLEWLGVIWSGGSTDYNAAFISRLSISKDNSKSQVFFKMNSLQADDTAIYYCARNYGYDYAMDYWGQGTSVTVSS

SEQ ID NO: 32 - protein, 107 aa, Artificial Sequence
  Synthetic: light chain variable region sequence
DILLTQSPAILSVSPGERVSFSCRASQSIGTSIHWYQQRTNGSPRLLIKYASESISGIPSRFSGSGSGTDFTLSINSVESEDIADYYCQQSNSWPFTFGSGTKLEIK

SEQ ID NO: 33 - protein, 10 aa, Artificial Sequence
  Synthetic: heavy chain variable region CDR1 of the anti-ceramide antibody
GYTFTNYWMH

SEQ ID NO: 34 - protein, 17 aa, Artificial Sequence
  Synthetic: heavy chain variable region CDR2
AIYPGDSDTSYNQKFKG

SEQ ID NO: 35 - protein, 7 aa, Artificial Sequence
  Synthetic: heavy chain variable region CDR3
GLYYGYD

SEQ ID NO: 36 - protein, 16 aa, Artificial Sequence
  Synthetic: light chain variable region CDR1
KSSQSLIDSDGKTFLN

SEQ ID NO: 37 - protein, 7 aa, Artificial Sequence
  Synthetic: light chain variable region CDR2
LVSKLDS

SEQ ID NO: 38 - protein, 9 aa, Artificial Sequence
  Synthetic: said light chain variable region CDR3
WQGTHFPYT

SEQ ID NO: 39 - protein, 115 aa, Artificial Sequence
  Synthetic: heavy chain variable region sequence comprising  the sequence
EVQLQQSGTVLARPGASVKMSCKASGYTFTNYWMHWVKQRPVQGLEWIGAIYPGDSDTSYNQKFKGKAKLTAVTSTSTAFMELSSLTNEDSAVYYCTGLYYGYDWGQGTTLTVSS

SEQ ID NO: 40 - protein, 112 aa, Artificial Sequence
  Synthetic: light chain variable region sequence
DVLMTQTPLTLSVTIGQPASISCKSSQSLIDSDGKTFLNWLLQRPGQSPKRLIYLVSKLDSGVPDRFTGSGSGTDFTLKISRVEAEDLGLYYCWQGTHFPYTFGGGTKLEIK

SEQ ID NO: 41 - protein, 109 aa, Homo sapiens
  misc_feature: human V gene 1-46
QVQLVQSGAEVKKPGASVKVSCKASGYTFTSYYMHWVRQAPGQGLEWMGIINPSGGSTSYAQKFQGRVTMTRDTSTSTVYMELSSLRSEDTAVYYCARWGQGTTVTVSS

SEQ ID NO: 42 - protein, 113 aa, Artificial Sequence
  Synthetic: VL 2A2
DVLMTQTPLTLSVTIGQPASISCKSSQSLIDSDGKTFLNWLLQRPGQSPKRLIYLVSKLDSGVPDRFTGSGSGTDFTLKISRVEAEDLGLYYCWQGTHFPYTFGGGTKLEIKR

SEQ ID NO: 43 - protein, 112 aa, Homo sapiens
  misc_feature: human V gene A1
DVVMTQSPLSLPVTLGQPASISCRSSQSLVYSDGNTYLNWFQQRPGQSPRRLIYKVSNWDSGVPDRFSGSGSGTDFTLKISRVEAEDVGVYYCMQGTHWPTFGQGTKLEIKR

SEQ ID NO: 44 - DNA, 1395 bp, Artificial Sequence
  Synthetic: Humanized 2A2 Heavy chain sequence
atggactggacctggagggtcttctgcttgctggctgtagctccaggtgctcactcccaggtgcagcttgtgcagtctggggctgaggtgaaaaagcctggggcttcagtgaaggtgtcctgcaaggcttctggctacacctttaccaactactggatgcactgggtaagacaggcgcctggacagggtctggaatggatgggcgctatttatcctggagatagtgatactagctacaaccagaagttcaagggccgggtcacaatgactcgagacacatccaccagcactgtctacatggagctcagcagcctgagaagtgaggacactgcggtctattactgtgcacgcctttactacggctacgactggggccaaggcaccactgtcacagtctcctcagccagcacgaagggcccatcggtcttccccctggcaccctcctccaagagcacctctgggggcacagcggccctgggctgcctggtcaaggactacttccccgaaccggtgacggtgtcgtggaactcaggcgccctgaccagcggcgtgcacaccttcccggctgtcctacagtcctcaggactctactccctcagcagcgtggtgaccgtgccctccagcagcttgggcacccagacctacatctgcaacgtgaatcacaagcccagcaacaccaaggtggacaagaaagttgagcccaaatcttgtgacaaaactcacacatgcccaccgtgcccagcacctgaactcctggggggaccgtcagtcttcctcttccccccaaaacccaaggacaccctcatgatctcccggacccctgaggtcacatgcgtggtggtggacgtgagccacgaagaccctgaggtcaagttcaactggtacgtggacggcgtggaggtgcataatgccaagacaaagccgcgggaggagcagtacaacagcacgtaccgtgtggtcagcgtcctcaccgtcctgcaccaggactggctgaatggcaaggagtacaagtgcaaggtctccaacaaagccctcccagcccccatcgagaaaaccatctccaaagccaaagggcagccccgagaaccacaggtgtacaccctgcccccatcccgggatgagctgaccaagaaccaggtcagcctgacctgcctggtcaaaggcttctatcccagcgacatcgccgtggagtgggagagcaatgggcagccggagaacaactacaagaccacgcctcccgtgctggactccgacggctccttcttcctctacagcaagctcaccgtggacaagagcaggtggcagcaggggaacgtcttctcatgctccgtgatgcatgaggctctgcacaaccactacacgcagaagagcctctccctgtccccgggtaaatga

SEQ ID NO: 45 - protein, 463 aa, Artificial Sequence
  Synthetic: Humanized 2A2 Heavy chain sequence
MDWTWRVFCLLAVAPGAHSQVQLVQSGAEVKKPGASVKVSCKASGYTFTNYWMHWVRQAPGQGLEWMGAIYPGDSDTSYNQKFKGRVTMTRDTSTSTVYMELSSLRSEDTAVYYCARLYYGYDWGQGTTVTVSSASTKGPSVFPLAPSSKSTSGGTAALGCLVKDYFPEPVTVSWNSGALTSGVHTFPAVLQSSGLYSLSSVVTVPSSSLGTQTYICNVNHKPSNTKVDKKVEPKSCDKTHTCPPCPAPELLGGPSVFLFPPKPKDTLMISRTPEVTCVVVDVSHEDPEVKFNWYVDGVEVHNAKTKPREEQYNSTYRVVSVLTVLHQDWLNGKEYKCKVSNKALPAPIEKTISKAKGQPREPQVYTLPPSRDELTKNQVSLTCLVKGFYPSDIAVEWESNGQPENNYKTTPPVLDSDGSFFLYSKLTVDKSRWQQGNVFSCSVMHEALHNHYTQKSLSLSPG